European Patent Specification EP 3 740 246 B9, published September 27, 2023. Title: Disrupting the LINC complex for treating Laminopathy. Applicant: Agency for Science, Technology and Research. The sequence listing filed with the application follows.

SEQUENCE LISTING (81 sequences)

SEQ ID NO: 1 - DNA, 15424 bp, Artificial Sequence
  Plasmid pAdDeltaF6
tcgacggtatcgataagcttgatatcgaattcctgcagcccgggggatccactagttctagagcggccgccaccgcggtggagctccagcttttgttccctttagtgagggttaatttcgagcttggcgtaatcatggtcatagctgtttcctgtgtgaaattgttatccgctcacaattccacacaacatacgagccggaagcataaagtgtaaagcctggggtgcctaatgagtgagctaactcacattaattgcgttgcgctcactgcccgctttccagtcgggaaacctgtcgtgccagctgcattaatgaatcggccaacgcgcggggagaggcggtttgcgtattgggcgctcttccgcttcctcgctcactgactcgctgcgctcggtcgttcggctgcggcgagcggtatcagctcactcaaaggcggtaatacggttatccacagaatcaggggataacgcaggaaagaacatgtgagcaaaaggccagcaaaaggccaggaaccgtaaaaaggccgcgttgctggcgtttttccataggctccgcccccctgacgagcatcacaaaaatcgacgctcaagtcagaggtggcgaaacccgacaggactataaagataccaggcgtttccccctggaagctccctcgtgcgctctcctgttccgaccctgccgcttaccggatacctgtccgcctttctcccttcgggaagcgtggcgctttctcatagctcacgctgtaggtatctcagttcggtgtaggtcgttcgctccaagctgggctgtgtgcacgaaccccccgttcagcccgaccgctgcgccttatccggtaactatcgtcttgagtccaacccggtaagacacgacttatcgccactggcagcagccactggtaacaggattagcagagcgaggtatgtaggcggtgctacagagttcttgaagtggtggcctaactacggctacactagaaggacagtatttggtatctgcgctctgctgaagccagttaccttcggaaaaagagttggtagctcttgatccggcaaacaaaccaccgctggtagcggtggtttttttgtttgcaagcagcagattacgcgcagaaaaaaaggatctcaagaagatcctttgatcttttctacggggtctgacgctcagtggaacgaaaactcacgttaagggattttggtcatgagattatcaaaaaggatcttcacctagatccttttaaattaaaaatgaagttttaaatcaatctaaagtatatatgagtaaacttggtctgacagttaccaatgcttaatcagtgaggcacctatctcagcgatctgtctatttcgttcatccatagttgcctgactccccgtcgtgtagataactacgatacgggagggcttaccatctggccccagtgctgcaatgataccgcgagacccacgctcaccggctccagatttatcagcaataaaccagccagccggaagggccgagcgcagaagtggtcctgcaactttatccgcctccatccagtctattaattgttgccgggaagctagagtaagtagttcgccagttaatagtttgcgcaacgttgttgccattgctacaggcatcgtggtgtcacgctcgtcgtttggtatggcttcattcagctccggttcccaacgatcaaggcgagttacatgatcccccatgttgtgcaaaaaagcggttagctccttcggtcctccgatcgttgtcagaagtaagttggccgcagtgttatcactcatggttatggcagcactgcataattctcttactgtcatgccatccgtaagatgcttttctgtgactggtgagtactcaaccaagtcattctgagaatagtgtatgcggcgaccgagttgctcttgcccggcgtcaatacgggataataccgcgccacatagcagaactttaaaagtgctcatcattggaaaacgttcttcggggcgaaaactctcaaggatcttaccgctgttgagatccagttcgatgtaacccactcgtgcacccaactgatcttcagcatcttttactttcaccagcgtttctgggtgagcaaaaacaggaaggcaaaatgccgcaaaaaagggaataagggcgacacggaaatgttgaatactcatactcttcctttttcaatattattgaagcatttatcagggttattgtctcatgagcggatacatatttgaatgtatttagaaaaataaacaaataggggttccgcgcacatttccccgaaaagtgccacctgacgtctaagaaaccattattatcatgacattaacctataaaaataggcgtatcacgaggccctttcgtcttcaagaattctcatgtttgacagcttatcatcgataagctttaatgcggtagtttatcacagttaaattgctaacgcagtcaggcaccgtgtatgaaatctaacaatgcgctcatcgtcatcctcggcaccgtcaccctggatgctgtaggcataggcttggttatgccggtactgccgggcctcttgcgggatatcgtccattccgacagcatcgccagtcactatggcgtgctgctagcgctatatgcgttgatgcaatttctatgcgcacccgttctcggagcactgtccgaccgctttggccgccgcccagtcctgctcgcttcgctacttggagccactatcgactacgcgatcatggcgaccacacccgtcctgtggatccggcgcacaccaaaaacgtcacttttgccacatccgtcgcttacatgtgttccgccacacttgcaacatcacacttccgccacactactacgtcacccgccccgttcccacgccccgcgccacgtcacaaactccaccccctcattatcatattggcttcaatccaaaataaatcatcaataatataccttattttggattgaagccaatatgataatgagggggtggagtttgtgacgtggcgcggggcgtgggaacggggcgggtgacgtaggttttagggcggagtaacttgtatgtgttgggaattgtagttttcttaaaatgggaagttacgtaacgtgggaaaacggaagtgacgatttgaggaagttgtgggttttttggctttcgtttctgggcgtaggttcgcgtgcggttttctgggtgttttttgtggactttaaccgttacgtcattttttagtcctatatatactcgctctgcacttggcccttttttacactgtgactgattgagctggtgccgtgtcgagtggtgtttttttaataggttttcttttttactggtaaggctgactgttaggctgccgctgtgaagcgctgtatgttgttctggagcgggagggtgctattttgcctaggcaggagggtttttcaggtgtttatgtgtttttctctcctattaattttgttatacctcctatgggggctgtaatgttgtctctacgcctgcgggtatgtattcccccgggctatttcggtcgctttttagcactgaccgatgaatcaacctgatgtgtttaccgagtcttacattatgactccggacatgaccgaggagctgtcggtggtgctttttaatcacggtgaccagtttttttacggtcacgccggcatggccgtagtccgtcttatgcttataagggttgtttttcctgttgtaagacaggcttctaatgtttaaatgtttttttgttattttattttgtgtttatgcagaaacccgcagacatgtttgagagaaaaatggtgtctttttctgtggtggttccggagcttacctgcctttatctgcatgagcatgactacgatgtgctttcttttttgcgcgaggctttgcctgattttttgagcagcaccttgcattttatatcgccgcccatgcaacaaagcttacatcggggctacgctggttagcatagctccgagtatgcgtgtcataatcagtgtgggttcttttgtcaaggttcctggcggggaagtggccgcgctggtccgtgcagacctgcacgattatgttcagctggccctgcgaagggacctacgggatcgcggtatttttgttaatgttccgcttttgaatcttatacaggtctgtgaggaacctgaatttttgcaatcatgattcgctgcttgaggctgaaggtggagggcgctctggagcagatttttacaatggccggacttaatattcgggatttgcttagagatatattgagaaggtggcgagatgagaattatttgggcatggttgaaggtgctggaatgtttatagaggagattcaccctgaagggtttagcctttacgtccacttggacgtgagggccgtttgccttttggaagccattgtgcaacatcttacaaatgccattatctgttctttggctgtagagtttgaccacgccaccggaggggagcgcgttcacttaatagatcttcattttgaggttttggataatcttttggaataaaaaaaaaaacatggttcttccagctcttcccgctcctcccgtgtgtgactcgcagaacgaatgtgtaggttggctgggtgtggcttattctgcggtggtggatgttatcagggcagcggcgcatgaaggagtttacatagaacccgaagccagggggcgcctggatgctttgagagagtggatatactacaactactacacagagcgatctaagcggcgagaccggagacgcagatctgtttgtcacgcccgcacctggttttgcttcaggaaatatgactacgtccggcgttccatttggcatgacactacgaccaacacgatctcggttgtctcggcgcactccgtacagtagggatcgtctacctccttttgagacagaaacccgcgctaccatactggaggatcatccgctgctgcccgaatgtaacactttgacaatgcacaacgtgagttacgtgcgaggtcttccctgcagtgtgggatttacgctgattcaggaatgggttgttccctgggatatggttctaacgcgggaggagcttgtaatcctgaggaagtgtatgcacgtgtgcctgtgttgtgccaacattgatatcatgacgagcatgatgatccatggttacgagtcctgggctctccactgtcattgttccagtcccggttccctgcagtgtatagccggcgggcaggttttggccagctggtttaggatggtggtggatggcgccatgtttaatcagaggtttatatggtaccgggaggtggtgaattacaacatgccaaaagaggtaatgtttatgtccagcgtgtttatgaggggtcgccacttaatctacctgcgcttgtggtatgatggccacgtgggttctgtggtccccgccatgagctttggatacagcgccttgcactgtgggattttgaacaatattgtggtgctgtgctgcagttactgtgctgatttaagtgagatcagggtgcgctgctgtgcccggaggacaaggcgccttatgctgcgggcggtgcgaatcatcgctgaggagaccactgccatgttgtattcctgcaggacggagcggcggcggcagcagtttattcgcgcgctgctgcagcaccaccgccctatcctgatgcacgattatgactctacccccatgtaggcgtggacttctccttcgccgcccgttaagcaaccgcaagttggacagcagcctgtggctcagcagctggacagcgacatgaacttaagtgagctgcccggggagtttattaatatcactgatgagcgtttggctcgacaggaaaccgtgtggaatataacacctaagaatatgtctgttacccatgatatgatgctttttaaggccagccggggagaaaggactgtgtactctgtgtgttgggagggaggtggcaggttgaatactagggttctgtgagtttgattaaggtacggtgatctgtataagctatgtggtggtggggctatactactgaatgaaaaatgacttgaaattttctgcaattgaaaaataaacacgttgaaacataacacaaacgattctttattcttgggcaatgtatgaaaaagtgtaagaggatgtggcaaatatttcattaatgtagttgtggccagaccagtcccatgaaaatgacatagagtatgcacttggagttgtgtctcctgtttcctgtgtaccgtttagtgtaatggttagtgttacaggtttagttttgtctccgtttaagtaaacttgactgacaatgttacttttggcagttttaccgtgagattttggataagctgataggttaggcataaatccaacagcgtttgtataggctgtgccttcagtaagatctccatttctaaagttccaatattctgggtccaggaaggaattgtttagtagcactccattttcgtcaaatcttataataagatgagcactttgaactgttccagatattggagccaaactgcctttaacagccaaaactgaaactgtagcaagtatttgactgccacattttgttaagaccaaagtgagtttagcatctttctctgcatttagtctacagttaggagatggagctggtgtggtccacaaagttagcttatcattatttttgtttcctactgtaatggcacctgtgctgtcaaaactaaggccagttcctagtttaggaaccatagccttgtttgaatcaaattctaggccatggccaatttttgttttgaggggatttgtgtttggtgcattaggtgaaccaaattcaagcccatctcctgcattaatggctatggctgtagcgtcaaacatcaaccccttggcagtgcttaggttaacctcaagctttttggaattgtttgaagctgtaaacaagtaaaggcctttgttgtagttaatatccaagttgtgggctgagtttataaaaagagggccctgtcctagtcttagatttagttggttttgagcatcaaacggataactaacatcaagtataaggcgtctgttttgagaatcaatccttagtcctcctgctacattaagttgcatattgccttgtgaatcaaaacccaaggctccagtaactttagtttgcaaggaagtattattaatagtcacacctggaccagttgctacggtcaaagtgtttaggtcgtctgttacatgcaaaggagccccgtactttagtcctagttttccattttgtgtataaatgggctctttcaagtcaatgcccaagctaccagtggcagtagttagagggggtgaggcagtgatagtaagggtactgctatcggtggtggtgagggggcctgatgtttgcagggctagctttccttctgacactgtgaggggtccttgggtggcaatgctaagtttggagtcgtgcacggttagcggggcctgtgattgcatggtgagtgtgttgcccgcgaccattagaggtgcggcggcagccacagttagggcttctgaggtaactgtgaggggtgcagatatttccaggtttatgtttgacttggtttttttgagaggtgggctcacagtggttacattttgggaggtaaggttgccggcctcgtccagagagaggccgttgcccattttgagcgcaagcatgccattggaggtaactagaggttcggataggcgcaaagagagtaccccagggggactctcttgaaacccattgggggatacaaagggaggagtaagaaaaggcacagttggaggaccggtttccgtgtcatatggatacacggggttgaaggtatcttcagacggtcttgcgcgcttcatctgcaacaacatgaagatagtgggtgcggatggacaggaacaggaggaaactgacattccatttagattgtggagaaagtttgcagccaggaggaagctgcaataccagagctgggaggagggcaaggaggtgctgctgaataaactggacagaaatttgctaactgattttaagtaagtgatgctttattatttttttttattagttaaagggaataagatccccgggtactctagttaattaactagaggatcttgatgtaatccaaggttaggacagttgcaaatcacagtgagaacacagggtcccctgtcccgctcaactagcagggggcgctgggtaaactcccgaatcaggctacgggcaagctctccctgggcggtaagccggacgccgtgcgccgggccctcgatatgatcctcgggcaattcaaagtagcaaaactcaccggagtcgcgggcaaagcacttgtggcggcgacagtggaccaggtgtttcaggcgcagttgctctgcctctccacttaacattcagtcgtagccgtccgccgagtcctttaccgcgtcaaagttaggaataaattgatccggatagtggccgggaggtcccgagaaggggttaaagtagaccgatggcacaaactcctcaataaattgcagagttccaatgcctccagagcgcggctcagaggacgaggtctgcagagttaggattgcctgacgaggcgtgaatgaaggacggccggcgccgccgatctgaaatgtcccgtccggacggagaccaagcgaggagctcaccgactcgtcgttgagctgaatacctcgccctctgattgtcaggtgagttataccctgcccgggcgaccgcaccctgtgacgaaagccgcccgcaagctgcgcccctgagttagtcatctgaacttcggcctgggcgtctctgggaagtaccacagtggtgggagcgggactttcctggtacaccagggcagcgggccaactacggggattaaggttattacgaggtgtggtggtaatagccgcctgttccaagagaattcggtttcggtgggcgcggattccgttgacccgggatatcatgtggggtcccgcgctcatgtagtttattcgggttgagtagtcttgggcagctccagccgcaagtcccatttgtggctggtaactccacatgtagggcgtgggaatttccttgctcataatggcgctgacgacaggtgctggcgccgggtgtggccgctggagatgacgtagttttcgcgcttaaatttgagaaagggcgcgaaactagtccttaagagtcagcgcgcagtatttactgaagagagcctccgcgtcttccagcgtgcgccgaagctgatcttcgcttttgtgatacaggcagctgcgggtgagggatcgcagagacctgttttttattttcagctcttgttcttggcccctgctctgttgaaatatagcatacagagtgggaaaaatcctgtttctaagctcgcgggtcgatacgggttcgttgggcgccagacgcagcgctcctcctcctgctgctgccgccgctgtggatttcttgggctttgtcagagtcttgctatccggtcgcctttgcttctgtgtggccgctgctgttgctgccgctgccgctgccgccggtgcagtatgggctgtagagatgacggtagtaatgcaggatgttacgggggaaggccacgccgtgatggtagagaagaaagcggcgggcgaaggagatgttgcccccacagtcttgcaagcaagcaactatggcgttcttgtgcccgcgccatgagcggtagccttggcgctgttgttgctcttgggctaacggcggcggctgcttggacttaccggccctggttccagtggtgtcccatctacggttgggtcggcgaacgggcagtgccggcggcgcctgaggagcggaggttgtagccatgctggaaccggttgccgatttctggggcgccggcgaggggaatgcgaccgagggtgacggtgtttcgtctgacacctcttcgacctcggaagcttcctcgtctaggctctcccagtcttccatcatgtcctcctcctcctcgtccaaaacctcctctgcctgactgtcccagtattcctcctcgtccgtgggtggcggcggcagctgcagcttctttttgggtgccatcctgggaagcaagggcccgcggctgctgctgatagggctgcggcggcggggggattgggttgagctcctcgccggactgggggtccaagtaaaccccccgtccctttcgtagcagaaactcttggcgggctttgttgatggcttgcaattggccaagaatgtggccctgggtaatgacgcaggcggtaagctccgcatttggcgggcgggattggtcttcgtagaacctaatctcgtgggcgtggtagtcctcaggtacaaatttgcgaaggtaagccgacgtccacagccccggagtgagtttcaaccccggagccgcggacttttcgtcaggcgagggaccctgcagctcaaaggtaccgataatttgactttcgttaagcagctgcgaattgcaaaccagggagcggtgcggggtgcataggttgcagcgacagtgacactccagtagaccgtcaccgctcacgtcttccattatgtcagagtggtaggcaaggtagttggctagctgcagaaggtagcagtggccccaaagcggcggagggcattcgcggtacttaatgggcacaaagtcgctaggaagtgcacagcaggtggcgggcaagattcctgagcgctctaggataaagttcctaaagttctgcaacatgctttgactggtgaagtctggcagaccctgttgcagggttttaagcaggcgttcggggaaaatgatgtccgccaggtgcgcggccacggagcgctcgttgaaggccgtccataggtccttcaagttttgctttagcagtttctgcagctccttgaggttgcactcctccaagcactgctgccaaacgcccatggccgtctgccaggtgtagcatagaaataagtaaacgcagtcgcggacgtagtcgcggcgcgcctcgcccttgagcgtggaatgaagcacgttttgcccaaggcggttttcgtgcaaaattccaaggtaggagaccaggttgcagagctccacgttggagatcttgcaggcctggcgtacgtagccctgtcgaaaggtgtagtgcaatgtttcctctagcttgcgctgcatctccgggtcagcaaagaaccgctgcatgcactcaagctccacggtaacgagcactgcggccatcattagtttgcgtcgctcctccaagtcggcaggctcgcgcgtttgaagccagcgcgctagctgctcgtcgccaactgcgggtaggccctcctctgtttgttcttgcaaatttgcatccctctccaggggctgcgcacggcgcacgatcagctcactcatgactgtgctcatgaccttggggggtaggttaagtgccgggtaggcaaagtgggtgacctcgatgctgcgttttagtacggctaggcgcgcgttgtcaccctcgagttccaccaacactccagagtgactttcattttcgctgttttcctgttgcagagcgtttgccgcgcgcttctcgtcgcgtccaagaccctcaaagatttttggcacttcgttgagcgaggcgatatcaggtatgacagcgccctgccgcaaggccagctgcttgtccgctcggctgcggttggcacggcaggataggggtatcttgcagttttggaaaaagatgtgataggtggcaagcacctctggcacggcaaatacggggtagaagttgaggcgcgggttgggctcgcatgtgccgttttcttggcgtttggggggtacgcgcggtgagaataggtggcgttcgtaggcaaggctgacatccgctatggcgaggggcacatcgctgcgctcttgcaacgcgtcgcagataatggcgcactggcgctgcagatgcttcaacagcacgtcgtctcccacatctaggtagtcgccatgcctttcgtccccccgcccgacttgttcctcgtttgcctctgcgttgtcctggtcttgctttttatcctctgttggtactgagcggtcctcgtcgtcttcgcttacaaaacctgggtcctgctcgataatcacttcctcctcctcaagcgggggtgcctcgacggggaaggtggtaggcgcgttggcggcatcggtggaggcggtggtggcgaactcagagggggcggttaggctgtccttcttctcgactgactccatgatctttttctgcctataggagaaggaaatggccagtcgggaagaggagcagcgcgaaaccacccccgagcgcggacgcggtgcggcgcgacgtcccccaaccatggaggacgtgtcgtccccgtccccgtcgccgccgcctccccgggcgcccccaaaaaagcggatgaggcggcgtatcgagtccgaggacgaggaagactcatcacaagacgcgctggtgccgcgcacacccagcccgcggccatcgacctcggcggcggatttggccattgcgcccaagaagaaaaagaagcgcccttctcccaagcccgagcgcccgccatcaccagaggtaatcgtggacagcgaggaagaaagagaagatgtggcgctacaaatggtgggtttcagcaacccaccggtgctaatcaagcatggcaaaggaggtaagcgcacagtgcggcggctgaatgaagacgacccagtggcgcgtggtatgcggacgcaagaggaagaggaagagcccagcgaagcggaaagtgaaattacggtgatgaacccgctgagtgtgccgatcgtgtctgcgtgggagaagggcatggaggctgcgcgcgcgctgatggacaagtaccacgtggataacgatctaaaggcgaacttcaaactactgcctgaccaagtggaagctctggcggccgtatgcaagacctggctgaacgaggagcaccgcgggttgcagctgaccttcaccagcaacaagacctttgtgacgatgatggggcgattcctgcaggcgtacctgcagtcgtttgcagaggtgacctacaagcatcacgagcccacgggctgcgcgttgtggctgcaccgctgcgctgagatcgaaggcgagcttaagtgtctacacggaagcattatgataaataaggagcacgtgattgaaatggatgtgacgagcgaaaacgggcagcgcgcgctgaaggagcagtctagcaaggccaagatcgtgaagaaccggtggggccgaaatgtggtgcagatctccaacaccgacgcaaggtgctgcgtgcacgacgcggcctgtccggccaatcagttttccggcaagtcttgcggcatgttcttctctgaaggcgcaaaggctcaggtggcttttaagcagatcaaggcttttatgcaggcgctgtatcctaacgcccagaccgggcacggtcaccttttgatgccactacggtgcgagtgcaactcaaagcctgggcacgcgccctttttgggaaggcagctaccaaagttgactccgttcgccctgagcaacgcggaggacctggacgcggatctgatctccgacaagagcgtgctggccagcgtgcaccacccggcgctgatagtgttccagtgctgcaaccctgtgtatcgcaactcgcgcgcgcagggcggaggccccaactgcgacttcaagatatcggcgcccgacctgctaaacgcgttggtgatggtgcgcagcctgtggagtgaaaacttcaccgagctgccgcggatggttgtgcctgagtttaagtggagcactaaacaccagtatcgcaacgtgtccctgccagtggcgcatagcgatgcgcggcagaacccctttgatttttaaacggcgcagacggcaagggtgggggtaaataatcacccgagagtgtacaaataaaagcatttgcctttattgaaagtgtctctagtacattatttttacatgtttttcaagtgacaaaaagaagtggcgctcctaatctgcgcactgtggctgcggaagtagggcgagtggcgctccaggaagctgtagagctgttcctggttgcgacgcagggtgggctgtacctggggactgttgagcatggagttgggtaccccggtaataaggttcatggtggggttgtgatccatgggagtttggggccagttggcaaaggcgtggagaaacatgcagcagaatagtccacaggcggccgagttgggcccctgtacgctttgggtggacttttccagcgttatacagcggtcgggggaagaagcaatggcgctacggcgcaggagtgactcgtactcaaactggtaaacctgcttgagtcgctggtcagaaaagccaaagggctcaaagaggtagcatgtttttgagtgcgggttccaggcaaaggccatccagtgtacgcccccagtctcggtccgagactcgaaccgggggtcccgcgactcaacccttggaaaataaccctccggctacagggagcgagccacttaatgctttcgctttccagcctaaccgcttacgctgcgcgcggccagtggccaaaaaagctagcgcagcagccgccgcgcctggaaggaagccaaaaggagcactcccccgttgtctgacgtcgcacacctgggttcgacacgcgggcggtaaccgcatggatcacggcggacggccggatacggggctcgaaccccggtcgtccgccatgatacccttgcgaatttatccaccagaccacggaagagtgcccgcttacaggctctccttttgcacggtagagcgtcaacgattgcgcgcgcctgaccggccagagcgtcccgaccatggagcactttttgccgctgcgcaacatctggaaccgcgtccgcgactttccgcgcgcctccaccaccgccgccggcatcacctggatgtccaggtacatctacggatatcatcgccttatgttggaagatctcgcccccggagccccggccaccctacgctggcccctctaccgccagccgccgccgcactttttggtgggataccagtacctggtgcggacttgcaacgactacgtatttgactcgagggcttactcgcgtctcaggtacaccgagctctcgcagccgggtcaccagaccgttaactggtccgttatggccaactgcacttacaccatcaacacgggcgcataccaccgctttgtggacatggatgacttccagtctaccctcacgcaggtgcagcaggccatattagccgagcgcgttgtcgccgacctagccctgcttcagccgatgaggggcttcggggtcacacgcatgggaggaagagggcgccacctacggccaaactccgccgccgccgcagcgatagatgcaagagatgcaggacaagaggaaggagaagaagaagtgccggtagaaaggctcatgcaagactactacaaagacctgcgccgatgtcaaaacgaagcctggggcatggccgaccgcctgcgcattcagcaggccggacccaaggacatggtgcttctg

SEQ ID NO: 2 - DNA, 7330 bp, Artificial Sequence
  Plasmid pAAV2_9
gtcgacggtatcgggggagctcgcagggtctccattttgaagcgggaggtttgaacgcgcagccgccatgccggggttttacgagattgtgattaaggtccccagcgaccttgacgagcatctgcccggcatttctgacagctttgtgaactgggtggccgagaaggaatgggagttgccgccagattctgacatggatctgaatctgattgagcaggcacccctgaccgtggccgagaagctgcagcgcgactttctgacggaatggcgccgtgtgagtaaggccccggaggctcttttctttgtgcaatttgagaagggagagagctacttccacatgcacgtgctcgtggaaaccaccggggtgaaatccatggttttgggacgtttcctgagtcagattcgcgaaaaactgattcagagaatttaccgcgggatcgagccgactttgccaaactggttcgcggtcacaaagaccagaaatggcgccggaggcgggaacaaggtggtggatgagtgctacatccccaattacttgctccccaaaacccagcctgagctccagtgggcgtggactaatatggaacagtatttaagcgcctgtttgaatctcacggagcgtaaacggttggtggcgcagcatctgacgcacgtgtcgcagacgcaggagcagaacaaagagaatcagaatcccaattctgatgcgccggtgatcagatcaaaaacttcagccaggtacatggagctggtcgggtggctcgtggacaaggggattacctcggagaagcagtggatccaggaggaccaggcctcatacatctccttcaatgcggcctccaactcgcggtcccaaatcaaggctgccttggacaatgcgggaaagattatgagcctgactaaaaccgcccccgactacctggtgggccagcagcccgtggaggacatttccagcaatcggatttataaaattttggaactaaacgggtacgatccccaatatgcggcttccgtctttctgggatgggccacgaaaaagttcggcaagaggaacaccatctggctgtttgggcctgcaactaccgggaagaccaacatcgcggaggccatagcccacactgtgcccttctacgggtgcgtaaactggaccaatgagaactttcccttcaacgactgtgtcgacaagatggtgatctggtgggaggaggggaagatgaccgccaaggtcgtggagtcggccaaagccattctcggaggaagcaaggtgcgcgtggaccagaaatgcaagtcctcggcccagatagacccgactcccgtgatcgtcacctccaacaccaacatgtgcgccgtgattgacgggaactcaacgaccttcgaacaccagcagccgttgcaagaccggatgttcaaatttgaactcacccgccgtctggatcatgactttgggaaggtcaccaagcaggaagtcaaagactttttccggtgggcaaaggatcacgtggttgaggtggagcatgaattctacgtcaaaaagggtggagccaagaaaagacccgcccccagtgacgcagatataagtgagcccaaacgggtgcgcgagtcagttgcgcagccatcgacgtcagacgcggaagcttcgatcaactacgcggacaggtaccaaaacaaatgttctcgtcacgtgggcatgaatctgatgctgtttccctgcagacaatgcgagagactgaatcagaattcaaatatctgcttcactcacggtgtcaaagactgtttagagtgctttcccgtgtcagaatctcaacccgtttctgtcgtcaaaaaggcgtatcagaaactgtgctacattcatcacatcatgggaaaggtgccagacgcttgcactgcttgcgacctggtcaatgtggacttggatgactgtgtttctgaacaataaatgacttaaaccaggtatggctgccgatggttatcttccagattggctcgaggacaaccttagtgaaggaattcgcgagtggtgggctttgaaacctggagcccctcaacccaaggcaaatcaacaacatcaagacaacgctcgaggtcttgtgcttccgggttacaaataccttggacccggcaacggactcgacaagggggagccggtcaacgcagcagacgcggcggccctcgagcacgacaaggcctacgaccagcagctcaaggccggagacaacccgtacctcaagtacaaccacgccgacgccgagttccaggagcggctcaaagaagatacgtcttttgggggcaacctcgggcgagcagtcttccaggccaaaaagaggcttcttgaacctcttggtctggttgaggaagcggctaagacggctcctggaaagaagaggcctgtagagcagtctcctcaggaaccggactcctccgcgggtattggcaaatcgggtgcacagcccgctaaaaagagactcaatttcggtcagactggcgacacagagtcagtcccagaccctcaaccaatcggagaacctcccgcagccccctcaggtgtgggatctcttacaatggcttcaggtggtggcgcaccagtggcagacaataacgaaggtgccgatggagtgggtagttcctcgggaaattggcattgcgattcccaatggctgggggacagagtcatcaccaccagcacccgaacctgggccctgcccacctacaacaatcacctctacaagcaaatctccaacagcacatctggaggatcttcaaatgacaacgcctacttcggctacagcaccccctgggggtattttgacttcaacagattccactgccacttctcaccacgtgactggcagcgactcatcaacaacaactggggattccggcctaagcgactcaacttcaagctcttcaacattcaggtcaaagaggttacggacaacaatggagtcaagaccatcgccaataaccttaccagcacggtccaggtcttcacggactcagactatcagctcccgtacgtgctcgggtcggctcacgagggctgcctcccgccgttcccagcggacgttttcatgattcctcagtacgggtatctgacgcttaatgatggaagccaggccgtgggtcgttcgtccttttactgcctggaatatttcccgtcgcaaatgctaagaacgggtaacaacttccagttcagctacgagtttgagaacgtacctttccatagcagctacgctcacagccaaagcctggaccgactaatgaatccactcatcgaccaatacttgtactatctctcaaagactattaacggttctggacagaatcaacaaacgctaaaattcagtgtggccggacccagcaacatggctgtccagggaagaaactacatacctggacccagctaccgacaacaacgtgtctcaaccactgtgactcaaaacaacaacagcgaatttgcttggcctggagcttcttcttgggctctcaatggacgtaatagcttgatgaatcctggacctgctatggccagccacaaagaaggagaggaccgtttctttcctttgtctggatctttaatttttggcaaacaaggaactggaagagacaacgtggatgcggacaaagtcatgataaccaacgaagaagaaattaaaactactaacccggtagcaacggagtcctatggacaagtggccacaaaccaccagagtgcccaagcacaggcgcagaccggctgggttcaaaaccaaggaatacttccgggtatggtttggcaggacagagatgtgtacctgcaaggacccatttgggccaaaattcctcacacggacggcaactttcacccttctccgctgatgggagggtttggaatgaagcacccgcctcctcagatcctcatcaaaaacacacctgtacctgcggatcctccaacggccttcaacaaggacaagctgaactctttcatcacccagtattctactggccaagtcagcgtggagatcgagtgggagctgcagaaggaaaacagcaagcgctggaacccggagatccagtacacttccaactattacaagtctaataatgttgaatttgctgttaatactgaaggtgtatatagtgaaccccgccccattggcaccagatacctgactcgtaatctgtaattgcttgttaatcaataaaccgtttaattcgtttcagttgaactttggtctctgcgaagggcgaattcgtttaaacctgcaggactagaggtcctgtattagaggtcacgtgagtgttttgcgacattttgcgacaccatgtggtcacgctgggtatttaagcccgagtgagcacgcagggtctccattttgaagcgggaggtttgaacgcgcagccgccaagccgaattctgcagatatccatcacactggcggccgctcgactagagcggccgccaccgcggtggagctccagcttttgttccctttagtgagggttaattgcgcgcttggcgtaatcatggtcatagctgtttcctgtgtgaaattgttatccgctcacaattccacacaacatacgagccggaagcataaagtgtaaagcctggggtgcctaatgagtgagctaactcacattaattgcgttgcgctcactgcccgctttccagtcgggaaacctgtcgtgccagctgcattaatgaatcggccaacgcgcggggagaggcggtttgcgtattgggcgctcttccgcttcctcgctcactgactcgctgcgctcggtcgttcggctgcggcgagcggtatcagctcactcaaaggcggtaatacggttatccacagaatcaggggataacgcaggaaagaacatgtgagcaaaaggccagcaaaaggccaggaaccgtaaaaaggccgcgttgctggcgtttttccataggctccgcccccctgacgagcatcacaaaaatcgacgctcaagtcagaggtggcgaaacccgacaggactataaagataccaggcgtttccccctggaagctccctcgtgcgctctcctgttccgaccctgccgcttaccggatacctgtccgcctttctcccttcgggaagcgtggcgctttctcatagctcacgctgtaggtatctcagttcggtgtaggtcgttcgctccaagctgggctgtgtgcacgaaccccccgttcagcccgaccgctgcgccttatccggtaactatcgtcttgagtccaacccggtaagacacgacttatcgccactggcagcagccactggtaacaggattagcagagcgaggtatgtaggcggtgctacagagttcttgaagtggtggcctaactacggctacactagaagaacagtatttggtatctgcgctctgctgaagccagttaccttcggaaaaagagttggtagctcttgatccggcaaacaaaccaccgctggtagcggtggtttttttgtttgcaagcagcagattacgcgcagaaaaaaaggatctcaagaagatcctttgatcttttctacggggtctgacgctcagtggaacgaaaactcacgttaagggattttggtcatgagattatcaaaaaggatcttcacctagatccttttaaattaaaaatgaagttttaaatcaatctaaagtatatatgagtaaacttggtctgacagttaccaatgcttaatcagtgaggcacctatctcagcgatctgtctatttcgttcatccatagttgcctgactccccgtcgtgtagataactacgatacgggagggcttaccatctggccccagtgctgcaatgataccgcgagacccacgctcaccggctccagatttatcagcaataaaccagccagccggaagggccgagcgcagaagtggtcctgcaactttatccgcctccatccagtctattaattgttgccgggaagctagagtaagtagttcgccagttaatagtttgcgcaacgttgttgccattgctacaggcatcgtggtgtcacgctcgtcgtttggtatggcttcattcagctccggttcccaacgatcaaggcgagttacatgatcccccatgttgtgcaaaaaagcggttagctccttcggtcctccgatcgttgtcagaagtaagttggccgcagtgttatcactcatggttatggcagcactgcataattctcttactgtcatgccatccgtaagatgcttttctgtgactggtgagtactcaaccaagtcattctgagaatagtgtatgcggcgaccgagttgctcttgcccggcgtcaatacgggataataccgcgccacatagcagaactttaaaagtgctcatcattggaaaacgttcttcggggcgaaaactctcaaggatcttaccgctgttgagatccagttcgatgtaacccactcgtgcacccaactgatcttcagcatcttttactttcaccagcgtttctgggtgagcaaaaacaggaaggcaaaatgccgcaaaaaagggaataagggcgacacggaaatgttgaatactcatactcttcctttttcaatattattgaagcatttatcagggttattgtctcatgagcggatacatatttgaatgtatttagaaaaataaacaaataggggttccgcgcacatttccccgaaaagtgccacctaaattgtaagcgttaatattttgttaaaattcgcgttaaatttttgttaaatcagctcattttttaaccaataggccgaaatcggcaaaatcccttataaatcaaaagaatagaccgagatagggttgagtgttgttccagtttggaacaagagtccactattaaagaacgtggactccaacgtcaaagggcgaaaaaccgtctatcagggcgatggcccactacgtgaaccatcaccctaatcaagttttttggggtcgaggtgccgtaaagcactaaatcggaaccctaaagggagcccccgatttagagcttgacggggaaagccggcgaacgtggcgagaaaggaagggaagaaagcgaaaggagcgggcgctagggcgctggcaagtgtagcggtcacgctgcgcgtaaccaccacacccgccgcgcttaatgcgccgctacagggcgcgtcccattcgccattcaggctgcgcaactgttgggaagggcgatcggtgcgggcctcttcgctattacgccagctggcgaaagggggatgtgctgcaaggcgattaagttgggtaacgccagggttttcccagtcacgacgttgtaaaacgacggccagtgagcgcgcgtaatacgactcactatagggcgaattgggtaccgggccccccctcgatcgag

SEQ ID NO: 3 - DNA, 5720 bp, Artificial Sequence
  Plasmid pENN.AAV.cTnT.PI.Sun1-dom-neg
ctgcgcgctcgctcgctcactgaggccgcccgggcaaagcccgggcgtcgggcgacctttggtcgcccggcctcagtgagcgagcgagcgcgcagagagggagtggccaactccatcactaggggttccttgtagttaatgattaacccgccatgctacttatctaccagggtaatggggatcctctagaactatagctagaattcgcccttacgggccccccctcgaggtcgggataaaagcagtctgggctttcacatgacagcatctggggctgcggcagagggtcgggtccgaagcgctgccttatcagcgccccagccctgggaggtgacagctggctggcttgtgtcagcccctcgggcactcacgtatctccgtccgacgggtttaaaatagcaaaactctgaggccacacaatagcttgggcttatatgggctcctgtgggggaagggggagcacggagggggccggggccgctgctgccaaaatagcagctcacaagtgttgcattcctctctgggcgccgggcacattcctgctggctctgcccgccccggggtgggcgccggggggaccttaaagcctctgccccccaaggagcccttcccagacagccgccggcacccaccgctccgtgggacgatccccgaagctctagagctttattgcggtagtttatcacagttaaattgctaacgcagtcagtgcttctgacacaacagtctcgaacttaagctgcagaagttggtcgtgaggcactgggcaggtaagtatcaaggttacaagacaggtttaaggagaccaatagaaactgggcttgtcgagacagagaagactcttgcgtttctgataggcacctattggtcttactgacatccactttgcctttctctccacaggtgtccactcccagttcaattacagctcttaaggctagagtacttaatacgactcactataggctagcctcgagaattcacgcgggccgccatgaagtgggtaacctttatttcccttctttttctctttagctcggcctattccaggggtgtgtttcgtcgagatgggcccgcttacccttacgatgtaccggattacgcactcgacgattccaagggcatgcatagacctggccctcttcccccgagcccacctccaaaggttgatcacaaggcttcccagtggcctcaggagagtgacatggggcagaaggtagcttctttgagtgcgcagtgccacaaccatgatgagagacttgcagagctgacagtcctgcttcagaaactacagatacgggtagaccaagtggatgacggcagggaagggctgtcactgtgggtcaagaatgtggttggacagcacctgcaggagatgggcaccatagaaccacctgatgctaagactgacttcatgactttccaccatgaccatgaagtgcgtctctccaacttggaagatgttcttagaaaactgacagaaaaatctgaggctatccagaaggagctggaagaaaccaagctgaaagcaggcagcagggatgaagagcagcccctccttgaccgtgtgcagcacctagaactggaactgaacctgttgaagtcacagctgtcagactggcagcatctgaagaccagctgtgagcaggctggggcccgcatccaggagactgtgcagctcatgttctctgaggatcagcagggcggttccctcgagtggctattagagaagctttcttctcggttcgtgagcaaggatgagctgcaggtgctcttacatgaccttgagctgaaactgctgcagaatatcacacaccacatcaccgtgacaggacaggccccgacatccgaggctattgtgtctgccgtgaatcaggcagggatttcaggaatcacagaagcgcaagcacatatcattgtgaacaatgctctgaagctgtactcccaagacaagacggggatggtggactttgctctggagtctggaggtggcagcatcctaagcactcggtgctctgagacctatgagaccaagacggcactgctgagcctgtttggggtcccactgtggtacttctcacagtcacctcgagtggtgatccagcccgacatctacccagggaattgctgggcgttcaaaggttcccaggggtacctggtggtgcggttgtccatgaagatctacccaaccacattcaccatggaacacattccaaagacactatcacccactggtaacatctccagtgcccccaaagactttgcagtctatggactggaaacggagtatcaagaagaggggcagcctctgggacggttcacctatgaccaggaaggagactcactccagatgttccacacactggaaagacctgaccaagccttccagatagtagagctccgggtcctgtccaactggggccaccctgagtacacttgcctctaccggttccgagtccacggagagcccatccagaaagatgagttgtagtaaggtacctctagagtcgacccgggcggcctcgaggacggggtgaactacgcctgaggatccgatctttttccctctgccaaaaattatggggacatcatgaagccccttgagcatctgacttctggctaataaaggaaatttattttcattgcaatagtgtgttggaattttttgtgtctctcactcggaagcaattcgttgatctgaatttcgaccacccataatacccattaccctggtagataagtagcatggcgggttaatcattaactacaaggaacccctagtgatggagttggccactccctctctgcgcgctcgctcgctcactgaggccgggcgaccaaaggtcgcccgacgcccgggctttgcccgggcggcctcagtgagcgagcgagcgcgcagccttaattaacctaattcactggccgtcgttttacaacgtcgtgactgggaaaaccctggcgttacccaacttaatcgccttgcagcacatccccctttcgccagctggcgtaatagcgaagaggcccgcaccgatcgcccttcccaacagttgcgcagcctgaatggcgaatgggacgcgccctgtagcggcgcattaagcgcggcgggtgtggtggttacgcgcagcgtgaccgctacacttgccagcgccctagcgcccgctcctttcgctttcttcccttcctttctcgccacgttcgccggctttccccgtcaagctctaaatcgggggctccctttagggttccgatttagtgctttacggcacctcgaccccaaaaaacttgattagggtgatggttcacgtagtgggccatcgccctgatagacggtttttcgccctttgacgttggagtccacgttctttaatagtggactcttgttccaaactggaacaacactcaaccctatctcggtctattcttttgatttataagggattttgccgatttcggcctattggttaaaaaatgagctgatttaacaaaaatttaacgcgaattttaacaaaatattaacgcttacaatttaggtggcacttttcggggaaatgtgcgcggaacccctatttgtttatttttctaaatacattcaaatatgtatccgctcatgagacaataaccctgataaatgcttcaataatattgaaaaaggaagagtatgagtattcaacatttccgtgtcgcccttattcccttttttgcggcattttgccttcctgtttttgctcacccagaaacgctggtgaaagtaaaagatgctgaagatcagttgggtgcacgagtgggttacatcgaactggatctcaacagcggtaagatccttgagagttttcgccccgaagaacgttttccaatgatgagcacttttaaagttctgctatgtggcgcggtattatcccgtattgacgccgggcaagagcaactcggtcgccgcatacactattctcagaatgacttggttgagtactcaccagtcacagaaaagcatcttacggatggcatgacagtaagagaattatgcagtgctgccataaccatgagtgataacactgcggccaacttacttctgacaacgatcggaggaccgaaggagctaaccgcttttttgcacaacatgggggatcatgtaactcgccttgatcgttgggaaccggagctgaatgaagccataccaaacgacgagcgtgacaccacgatgcctgtagcaatggcaacaacgttgcgcaaactattaactggcgaactacttactctagcttcccggcaacaattaatagactggatggaggcggataaagttgcaggaccacttctgcgctcggcccttccggctggctggtttattgctgataaatctggagccggtgagcgtgggtctcgcggtatcattgcagcactggggccagatggtaagccctcccgtatcgtagttatctacacgacggggagtcaggcaactatggatgaacgaaatagacagatcgctgagataggtgcctcactgattaagcattggtaactgtcagaccaagtttactcatatatactttagattgatttaaaacttcatttttaatttaaaaggatctaggtgaagatcctttttgataatctcatgaccaaaatcccttaacgtgagttttcgttccactgagcgtcagaccccgtagaaaagatcaaaggatcttcttgagatcctttttttctgcgcgtaatctgctgcttgcaaacaaaaaaaccaccgctaccagcggtggtttgtttgccggatcaagagctaccaactctttttccgaaggtaactggcttcagcagagcgcagataccaaatactgttcttctagtgtagccgtagttaggccaccacttcaagaactctgtagcaccgcctacatacctcgctctgctaatcctgttaccagtggctgctgccagtggcgataagtcgtgtcttaccgggttggactcaagacgatagttaccggataaggcgcagcggtcgggctgaacggggggttcgtgcacacagcccagcttggagcgaacgacctacaccgaactgagatacctacagcgtgagctatgagaaagcgccacgcttcccgaagggagaaaggcggacaggtatccggtaagcggcagggtcggaacaggagagcgcacgagggagcttccagggggaaacgcctggtatctttatagtcctgtcgggtttcgccacctctgacttgagcgtcgatttttgtgatgctcgtcaggggggcggagcctatggaaaaacgccagcaacgcggcctttttacggttcctggccttttgctggccttttgctcacatgttctttcctgcgttatcccctgattctgtggataaccgtattaccgcctttgagtgagctgataccgctcgccgcagccgaacgaccgagcgcagcgagtcagtgagcgaggaagcggaagagcgcccaatacgcaaaccgcctctccccgcgcgttggccgattcattaatgcagctggcacgacaggtttcccgactggaaagcgggcagtgagcgcaacgcaattaatgtgagttagctcactcattaggcaccccaggctttacactttatgcttccggctcgtatgttgtgtggaattgtgagcggataacaatttcacacaggaaacagctatgaccatgattacgccagatttaattaaggccttaattagg

SEQ ID NO: 4 - DNA, 1461 bp, Artificial Sequence
  Humanized Sun1DN
  Start codon (1)..(3)
  Signal sequence (4)..(84)
  Sun1 (88)..(1446)
  KDEL (1447)..(1458)
  Stop codon (1459)..(1461)
atgaagtgggtaacctttatttcccttctttttctctttagctcggcctattccaggggtgtgtttcgtcgagatgggcccgctctcgatgacccccaggacgtgtttaaacccacgacttctcgcctgaagcagcctctgcagggtgacagtgaggcttttccgtggcattggatgagtggcgtggagcagcaggtggcctctctgtctggacagtgccaccaccatggtgagaatctccgagagctgaccactttgctacagaagctgcaggctcgggtggaccagatggaaggcggcgctgccgggccgtcagcttcggtcagagacgctgtgggacagcccccgagggagactgactttatggcctttcaccaagaacatgaagtgcgtatgtcacacttggaagatattctgggaaaactgagagaaaaatctgaggccatccagaaggaactagaacagaccaagcaaaaaacaatcagtgcggttggtgagcagctcctgcccacagtcgagcacctccagctggagctggatcagctaaagtcagagctgtccagctggcgacacgtgaagaccggctgtgagacagtggatgccgtacaagaaagagtggacgtgcaagtcagagaaatggtgaaactcctgttttccgaagatcagcaaggcggttctctggaacagctgctgcagaggttctcatcacagtttgtgagcaaaggcgacttgcagacgatgctgcgagacctgcagctgcagatcctgcggaacgtcacccaccacgtttccgtgaccaagcagctcccaacctcagaagccgtggtgtctgctgtgagcgaggcgggggcgtctggaataacagaggcgcaagcacgtgccatcgtgaacagcgccttgaagctgtattcccaagataagaccgggatggtggactttgctctggaatctggtggtggcagcatcttgagtactcgctgttctgaaacttacgaaaccaaaacggcgctgatgagtctgtttgggatcccgctgtggtacttctcgcagtccccgcgcgtggtcatccagcctgacatttaccccggtaactgctgggcatttaaaggctcccaggggtacctggtggtgaggctctccatgatgatccacccagccgccttcactctggagcacatccctaagacgctgtcgccaacaggcaacatcagcagcgcccccaaggacttcgccgtctatggattagaaaatgagtatcaggaagaagggcagcttctgggacagttcacgtatgatcaggatggggagtcgctccagatgttccaggccctgaaaagacccgacgacacagctttccaaatagtggaacttcggattttttctaactggggccatcctgagtatacctgtctgtatcggttcagagttcatggcgaacctgtcaagaaagatgagttgtga

SEQ ID NO: 5 - DNA, 1482 bp, Artificial Sequence
  SUN2
  Start codon (1)..(3)
  Signal sequence (4)..(84)
  Sun2 (88)..(1467)
  KDEL (1468)..(1479)
  Stop codon (1480)..(1482)
atgaagtgggtaacctttatttcccttctttttctctttagctcggcctattccaggggtgtgtttcgtcgagatgggcccgctctcgatgagggctgggaagccagagactcatcgccacatttccaggctgagcagcgtgttatgtcccgggtacactctctggagcggcgtctggaagctcttgctgctgaattttcctccaactggcagaaggaggccatgcggctggaacgtctggagctgcggcaaggggctcctggccagggaggtggtggtggcctgagccacgaggacaccctggcgctgctggaggggctagtgagccgccgtgaagctgccctgaaggaggatttccgcagggaaactgctgctcgcatccaggaagaactgtctgccctgagagcagagcatcagcaagactcagaagacctcttcaagaagatcgtccgggcctcccaggagtccgaggctcgcatccagcagctgaagtcagagtggcaaagcatgacccaggagtccttccaggagagctctgtgaaggagctgaggcggctggaggaccagctggccggcctgcagcaggagctggcggctctggcactgaagcagagctcggtggcggaagaagtgggcctgctgccccagcagatccaggccgtgcgggacgacgtggaatctcagttcccggcctggatcagtcagttccttgcccgaggtggagggggccgcgtggggctccttcagagagaggagatgcaagctcagctgcgagagctggagagcaagatcctcacccatgtggcagagatgcagggcaagtcggccagggaagccgcggcctccctgagcctgacgctgcagaaagaaggtgtgattggagtgacagaggagcaggtgcaccacatcgtgaagcaggccctgcagcgctacagtgaggaccgcatcgggctggcagactacgccctggagtcaggaggggccagcgtcatcagcacccgatgttctgagacctacgagaccaagacggccctcctcagcctcttcggcatccccctgtggtaccactcccagtcaccccgagtcatcctccagccagatgtgcacccaggcaactgctgggccttccaggggccacaaggcttcgccgtggtccgcctctctgcccgcatccgccccacagccgttaccttagagcatgtgcccaaggccttgtcacccaacagcactatctccagtgcccccaaggacttcgccatctttgggtttgacgaagacctgcagcaggaggggacactccttggcaagttcacttacgatcaggacggcgagcctattcagacgtttcactttcaggcccctacgatggccacgtaccaggtggtggagctgcggatcctgactaactggggccaccccgagtacacctgcatctaccgcttcagagtgcatggggagcccgcccacaaagatgagttgtag

SEQ ID NO: 6 - DNA, 180 bp, Artificial Sequence
  KASH1, derived from Nesprin-1
cgcggcttcctgttcagagtcctccgagcagctcttccccttcagcttctcctgctcctcctcatcgggcttgcctgccttgtaccaatgtcagaggaagactacagctgtgccctctccaacaactttgcccggtcattccaccccatgctcagatacacgaatggccctcctccactc

SEQ ID NO: 7 - protein, 60 aa, Artificial Sequence
  KASH1 amino acid sequence
RGFLFRVLRAALPLQLLLLLLIGLACLVPMSEEDYSCALSNNFARSFHPMLRYTNGPPPL

SEQ ID NO: 8 - DNA, 180 bp, Artificial Sequence
  KASH2, derived from Nesprin-2
cgctccttcctctcaagggtggtccgggcagccctacccctgcagctgctcctcctgctgctgctgctcctggcctgcctgctgccctcctccgaagaagactacagctgcactcaggccaacaactttgcccggtccttttaccccatgctgaggtacaccaatgggccaccccccaca

SEQ ID NO: 9 - protein, 60 aa, Artificial Sequence
  KASH2 amino acid sequence
RSFLSRVVRAALPLQLLLLLLLLLACLLPSSEEDYSCTQANNFARSFYPMLRYTNGPPPT

SEQ ID NO: 10 - DNA, 177 bp, Artificial Sequence
  KASH3, derived from Nesprin-3
ggctccctcttccggagggcgtgctgtgtggcgctcccactgcagctgcttctgctgctgttcctcctcctgctgttcctgctcccaatcagggaagaggaccgcagctgcaccctggccaacaacttcgcccgctccttcacgctcatgctgcgctacaatggcccaccacccacc

SEQ ID NO: 11 - protein, 59 aa, Artificial Sequence
  KASH3 amino acid sequence
GSLFRRACCVALPLQLLLLLFLLLLFLLPIREEDRSCTLANNFARSFTLMLRYNGPPPT

SEQ ID NO: 12 - DNA, 174 bp, Artificial Sequence
  KASH4, derived from Nesprin-4
gatcctgcatccaggcagcctctgaccttcctccttatcctcttcctcctcttcctcctcctggtgggtgccatgtttctcctgcccgcgtcaggaggcccctgctgctctcatgcccgaatacccaggacaccctacctggtgctcagctatgtcaatggtcttcccccagtc

SEQ ID NO: 13 - protein, 58 aa, Artificial Sequence
  KASH4 amino acid sequence
DPASRQPLTFLLILFLLFLLLVGAMFLLPASGGPCCSHARIPRTPYLVLSYVNGLPPV

SEQ ID NO: 14 - DNA, 144 bp, Artificial Sequence
  KASH5, derived from CCDC155/KASH5
ctcagagtcactcgacatccactgatcccagctcctgtcctgggcctgctgctgctgctgctgctctctgtcctgctgcttggcccgtccccacctcccacctggccccacctccagctctgctacctccagccccctccagtg

SEQ ID NO: 15 - protein, 48 aa, Artificial Sequence
  KASH5 amino acid sequence
LRVTRHPLIPAPVLGLLLLLLLSVLLLGPSPPPTWPHLQLCYLQPPPV

SEQ ID NO: 16 - DNA, 22 bp, Artificial Sequence
  FLX/FLX-F1 primer
ccagcttacagagcaccgagct

SEQ ID NO: 17 - DNA, 22 bp, Artificial Sequence
  FLX/FLX-F2 primer
tccttgcagtccctcttgcatc

SEQ ID NO: 18 - DNA, 21 bp, Artificial Sequence
  FLX/FLX-R1 primer
aggcaccattgtcacagggtc

SEQ ID NO: 19 - DNA, 29 bp, Artificial Sequence
  Sun1-F primer
ggcaagtggatctcttgtgaattcttgac

SEQ ID NO: 20 - DNA, 27 bp, Artificial Sequence
  Sun1-R primer
gtagcacccaccttggtgagctggtac

SEQ ID NO: 21 - DNA, 20 bp, Artificial Sequence
  Sun1-E8 primer
agccacataaccacctggag

SEQ ID NO: 22 - DNA, 26 bp, Artificial Sequence
  MyHC-tF primer
atgacagacagatccctcctatctcc

SEQ ID NO: 23 - DNA, 24 bp, Artificial Sequence
  MyHC-tR primer
ctcatcactcgttgcatcatcgac

SEQ ID NO: 24 - DNA, 20 bp, Artificial Sequence
  MyHC-F primer
caaatgttgcttgtctggtg

SEQ ID NO: 25 - DNA, 20 bp, Artificial Sequence
  MyHC-R primer
gtcagtcgagtgcacagttt

SEQ ID NO: 26 - DNA, 20 bp, Artificial Sequence
  mcm-3798t primer
aggtggacctgatcatggag

SEQ ID NO: 27 - DNA, 20 bp, Artificial Sequence
  mcm-8346t primer
ataccggagatcatgcaagc

SEQ ID NO: 28 - DNA, 24 bp, Artificial Sequence
  mcm-7338 primer
ctaggccacagaattgaaagatct

SEQ ID NO: 29 - DNA, 25 bp, Artificial Sequence
  mcm-7339 primer
gtaggtggaaattctagcatcatcc

SEQ ID NO: 30 - DNA, 44 bp, Artificial Sequence
  aav Sun1 F primer
cgagaattcacgcgggccgccatgaagtgggtaacctttatttc

SEQ ID NO: 31 - DNA, 46 bp, Artificial Sequence
  aav Sun1 R primer
cgggtcgactctagaggtaccttactacaactcatctttctggatg

SEQ ID NO: 32 - DNA, 44 bp, Artificial Sequence
  aav GFP Sun R primer
cgggtcgactctagaggtacttactacaactcatctttggatcc

SEQ ID NO: 33 - DNA, 21 bp, Artificial Sequence
  Sun1 delSUN RNA guide sequence
gcacaatagcctcggatgtcg

SEQ ID NO: 34 - DNA, 20 bp, Artificial Sequence
  Syne1-stop guide RNA sequence
ccgttggtatatctgagcat

SEQ ID NO: 35 - DNA, 21 bp, Artificial Sequence
  Tyrosinase4a guide RNA sequence
ggttatggccgataggtgcat

SEQ ID NO: 36 - DNA, 20 bp, Artificial Sequence
  Common reverse primer for in vitro transcription
aaaagcaccgactcggtgcc

SEQ ID NO: 37 - DNA, 39 bp, Artificial Sequence
  Sun1delSUN gRNA-specific forward primer
ttaatacgactcactatagcacaatagcctcggatgtcg

SEQ ID NO: 38 - DNA, 39 bp, Artificial Sequence
  Syne1-stop gRNA-specific forward primer
ttaatacgactcactatagccgttggtatatctgagcat

SEQ ID NO: 39 - DNA, 39 bp, Artificial Sequence
  Tyrosinase4a gRNA-specific forward primer
ttaatacgactcactataggttatggccgataggtgcat

SEQ ID NO: 40 - DNA, 20 bp, Artificial Sequence
  Syne1CT' del8 forward primer
tgctcctgctgctgcttatt

SEQ ID NO: 41 - DNA, 22 bp, Artificial Sequence
  Syne1CT' del8 reverse primer
acatggtggagcatttgtctcc

SEQ ID NO: 42 - DNA, 20 bp, Artificial Sequence
  Sun1 CRISPR forward primer
tgaccttgagctgaaactgc

SEQ ID NO: 43 - DNA, 20 bp, Artificial Sequence
  Sun1 CRISPR reverse primer
tcagaacactggcacacaca

SEQ ID NO: 44 - DNA, 20 bp, Artificial Sequence
  Potential guide RNA sequence, SYNE1
tcgtgtatctgagcatgggg

SEQ ID NO: 45 - DNA, 20 bp, Artificial Sequence
  Potential guide RNA sequence, SYNE1
gccattcgtgtatctgagca

SEQ ID NO: 46 - DNA, 20 bp, Artificial Sequence
  Potential guide RNA sequence, SYNE1
tccaccccatgctcagatac

SEQ ID NO: 47 - DNA, 20 bp, Artificial Sequence
  Potential guide RNA sequence, SYNE1
gagcatggggtggaatgacc

SEQ ID NO: 48 - DNA, 20 bp, Artificial Sequence
  Potential guide RNA sequence, SYNE1
tgagcatggggtggaatgac

SEQ ID NO: 49 - DNA, 20 bp, Artificial Sequence
  Potential guide RNA sequence, SYNE1
tcgtgtatctgagcatgggg

SEQ ID NO: 50 - DNA, 20 bp, Artificial Sequence
  Potential guide RNA sequence, SYNE1
cattcgtgtatctgagcatg

SEQ ID NO: 51 - DNA, 20 bp, Artificial Sequence
  Potential guide RNA sequence, SYNE1
ccattcgtgtatctgagcat

SEQ ID NO: 52 - DNA, 20 bp, Artificial Sequence
  Potential guide RNA sequence, SYNE1
gccattcgtgtatctgagca

SEQ ID NO: 53 - DNA, 20 bp, Artificial Sequence
  Potential guide RNA sequence, SYNE1
cccatgctcagatacacgaa

SEQ ID NO: 54 - DNA, 20 bp, Artificial Sequence
  Potential guide RNA sequence, SYNE1
cccggtcattccaccccatg

SEQ ID NO: 55 - DNA, 20 bp, Artificial Sequence
  Potential guide RNA sequence, SUN1
tttttctaactggggccatc

SEQ ID NO: 56 - DNA, 20 bp, Artificial Sequence
  Potential guide RNA sequence, SUN1
ccgatacagacaggtatact

SEQ ID NO: 57 - DNA, 20 bp, Artificial Sequence
  Potential guide RNA sequence, SUN1
aacttcggattttttctaac

SEQ ID NO: 58 - DNA, 20 bp, Artificial Sequence
  Potential guide RNA sequence, SUN1
acttcggattttttctaact

SEQ ID NO: 59 - DNA, 20 bp, Artificial Sequence
  Potential guide RNA sequence, SUN1
cttcggattttttctaactg

SEQ ID NO: 60 - DNA, 20 bp, Artificial Sequence
  Potential guide RNA sequence, SUN1
acagacaggtatactcagga

SEQ ID NO: 61 - DNA, 20 bp, Artificial Sequence
  Potential guide RNA sequence, SUN1
ctgagtatacctgtctgtat

SEQ ID NO: 62 - DNA, 20 bp, Artificial Sequence
  Potential guide RNA sequence, SUN1
ttctaactggggccatcctg

SEQ ID NO: 63 - DNA, 20 bp, Artificial Sequence
  Potential guide RNA sequence, SUN1
tctaactggggccatcctga

SEQ ID NO: 64 - DNA, 20 bp, Artificial Sequence
  Potential guide RNA sequence, SUN1
ctaactggggccatcctgag

SEQ ID NO: 65 - DNA, 20 bp, Artificial Sequence
  Potential guide RNA sequence, SUN1
taactggggccatcctgagt

SEQ ID NO: 66 - DNA, 21 bp, Artificial Sequence
  Cas9 mRNA and gRNA targeting SUN1 domain
gcacaatagcctcggatgtcg

SEQ ID NO: 67 - DNA, 20 bp, Artificial Sequence
  Cas9 mRNA and gRNA targeting the KASH1 domain
ccgttggtatatctgagcat

SEQ ID NO: 68 - DNA, 21 bp, Artificial Sequence
  gRNA targeting tyrosinase
ggttatggccgataggtgcat

SEQ ID NO: 69 - DNA, 176 bp, Mus musculus
catgaccttgagctgaaactgctgcagaatatcacacaccacatcaccgtgacaggacaggccccgacatccgaggctattgtgtctgccgtgaatcaggcagggatttcaggaatcacagaagcgcaagcacatatcattgtgaacaatgctctgaagctgtactcccaagacaa

SEQ ID NO: 70 - DNA, 180 bp, Artificial Sequence
  Sun1_plus4
catgaccttgagctgaaactgctgcagaatatcacacaccacatcaccgtgacaggacaggccccgagacacatccgaggctattgtgtctgccgtgaatcaggcagggatttcaggaatcacagaagcgcaagcacatatcattgtgaacaatgctctgaagctgtactcccaagacaa

SEQ ID NO: 71 - DNA, 169 bp, Artificial Sequence
  Sun1_del7
catgaccttgagctgaaactgctgcagaatatcacacaccacatcaccgtgacaggacaggccccgaggctattgtgtctgccgtgaatcaggcagggatttcaggaatcacagaagcgcaagcacatatcattgtgaacaatgctctgaagctgtactcccaagacaa

SEQ ID NO: 72 - protein, 253 aa, Mus musculus
WLLEKLSSRFVSKDELQVLLHDLELKLLQNITHHITVTGQAPTSEAIVSAVNQAGISGITEAQAHIIVNNALKLYSQDKTGMVDFALESGGGSILSTRCSETYETKTALLSLFGVPLWYFSQSPRVVIQPDIYPGNCWAFKGSQGYLVVRLSMKIYPTTFTMEHIPKTLSPTGNISSAPKDFAVYGLETEYQEEGQPLGRFTYDQEGDSLQMFHTLERPDQAFQIVELRVLSNWGHPEYTCLYRFRVHGEPIQ

SEQ ID NO: 73 - protein, 101 aa, Artificial Sequence
  Sun1_plus4 protein
WLLEKLSSRFVSKDELQVLLHDLELKLLQNITHHITVTGQAPRHIRGYCVCRESGRDFRNHRSASTYHCEQCSEAVLPRQDGDGGLCSGVWRWQHPKHSVL

SEQ ID NO: 74 - protein, 48 aa, Artificial Sequence
  Sun1_del7 protein
WLLEKLSSRFVSKDELQVLLHDLELKLLQNITHHITVTGQAPRLLCLP

SEQ ID NO: 75 - DNA, 180 bp, Mus musculus
tattggactcacctgccttgtacccatgtcagagaaagactacagctgtgccctctccaacaactttgcccgatccttccatccgatgctcagatataccaacggtcctcctccactctgaagcaagcagacatccccacacaagtgcaggcagtaagaggagaaggaatatcaaatggc

SEQ ID NO: 76 - DNA, 172 bp, Artificial Sequence
  Syne1_CTdel8
tattggactcacctgccttgtacccatgtcagagaaagactacagctgtgccctctccaacaactttgcccgatccttccatccgatataccaacggtcctcctccactctgaagcaagcagacatccccacacaagtgcaggcagtaagaggagaaggaatatcaaatggc

SEQ ID NO: 77 - protein, 79 aa, Mus musculus
STRDGSDSSRSDPRPERVGRAFLFRILRAALPFQLLLLLLIGLTCLVPMSEKDYSCALSNNFARSFHPMLRYTNGPPPL

SEQ ID NO: 78 - protein, 129 aa, Artificial Sequence
  Nesprin1_CTdel8
STRDGSDSSRSDPRPERVGRAFLFRILRAALPFQLLLLLLIGLTCLVPMSEKDYSCALSNNFARSFHPIYQRSSSTLKQADIPTQVQAVRGEGISNGREAPKEKFNILNHQGNANQNNPEMETNAPPCS

SEQ ID NO: 79 - DNA, 183 bp, Homo sapiens
cgcggcttcctgttcagagtcctccgagcagctcttccccttcagcttctcctgctcctcctcatcgggcttgcctgccttgtaccaatgtcagaggaagactacagctgtgccctctccaacaactttgcccggtcattccaccccatgctcagatacacgaatggccctcctccactctga

SEQ ID NO: 80 - DNA, 534 bp, Homo sapiens
gataagaccgggatggtggactttgctctggaatctggtggtggcagcatcttgagtactcgctgttctgaaacttacgaaaccaaaacggcgctgatgagtctgtttgggatcccgctgtggtacttctcgcagtccccgcgcgtggtcatccagcctgacatttaccccggtaactgctgggcatttaaaggctcccaggggtacctggtggtgaggctctccatgatgatccacccagccgccttcactctggagcacatccctaagacgctgtcgccaacaggcaacatcagcagcgcccccaaggacttcgccgtctatggattagaaaatgagtatcaggaagaagggcagcttctgggacagttcacgtatgatcaggatggggagtcgctccagatgttccaggccctgaaaagacccgacgacacagctttccaaatagtggaacttcggattttttctaactggggccatcctgagtatacctgtctgtatcggttcagagttcatggcgaacctgtcaagtga

SEQ ID NO: 81 - DNA, 117 bp, Homo sapiens
aaaagacccgacgacacagctttccaaatagtggaacttcggattttttctaactggggccatcctgagtatacctgtctgtatcggttcagagttcatggcgaacctgtcaagtga